European Patent Application EP 4 151 236 A1, published March 22, 2023. Title: A composition for treating or preventing obesity associated disease containing amphiregulin specific double stranded oligonucleotide structure. Applicant: BIONEER CORPORATION siRNAgen Therapeutics Corporation. The sequence listing filed with the application follows.

SEQUENCE LISTING (60 sequences)

SEQ ID NO: 1 - DNA, 19 bp, Artificial Sequence
  Amphiregulin siRNA sense
cctataaagcggcaggtgc

SEQ ID NO: 2 - DNA, 19 bp, Artificial Sequence
  Amphiregulin siRNA sense
gagcggcgcacactcccgg

SEQ ID NO: 3 - DNA, 19 bp, Artificial Sequence
  Amphiregulin siRNA sense
gtcccagagaccgagttgc

SEQ ID NO: 4 - DNA, 19 bp, Artificial Sequence
  Amphiregulin siRNA sense
gagacgccgccgctgcgaa

SEQ ID NO: 5 - DNA, 19 bp, Artificial Sequence
  Amphiregulin siRNA sense
ccggcgccggtggtgctgt

SEQ ID NO: 6 - DNA, 19 bp, Artificial Sequence
  Amphiregulin siRNA sense
ggtggtgctgtcgctcttg

SEQ ID NO: 7 - DNA, 19 bp, Artificial Sequence
  Amphiregulin siRNA sense
cgctcttgatactcggctc

SEQ ID NO: 8 - DNA, 19 bp, Artificial Sequence
  Amphiregulin siRNA sense
tcttgatactcggctcagg

SEQ ID NO: 9 - DNA, 19 bp, Artificial Sequence
  Amphiregulin siRNA sense
ggacctcaatgacacctac

SEQ ID NO: 10 - DNA, 19 bp, Artificial Sequence
  Amphiregulin siRNA sense
cacctactctgggaagcgt

SEQ ID NO: 11 - DNA, 19 bp, Artificial Sequence
  Amphiregulin siRNA sense
acctactctgggaagcgtg

SEQ ID NO: 12 - DNA, 19 bp, Artificial Sequence
  Amphiregulin siRNA sense
ctgggaagcgtgaaccatt

SEQ ID NO: 13 - DNA, 19 bp, Artificial Sequence
  Amphiregulin siRNA sense
gaagcgtgaaccattttct

SEQ ID NO: 14 - DNA, 19 bp, Artificial Sequence
  Amphiregulin siRNA sense
ttctggggaccacagtgct

SEQ ID NO: 15 - DNA, 20 bp, Artificial Sequence
  hGAPDH-F primer
ggtgaaggtcggagtcaacg

SEQ ID NO: 16 - DNA, 25 bp, Artificial Sequence
  hGAPDH-R primer
accatgtagttgaggtcaatgaagg

SEQ ID NO: 17 - DNA, 20 bp, Artificial Sequence
  hAREG F primer
acacctactctgggaagcgt

SEQ ID NO: 18 - DNA, 20 bp, Artificial Sequence
  hAREG R primer
gccaggtatttgtggttcgt

SEQ ID NO: 19 - DNA, 19 bp, Artificial Sequence
  mAmphiregulin siRNA sense strand
aacgggactgtgcatgcca

SEQ ID NO: 20 - DNA, 19 bp, Artificial Sequence
  mAmphiregulin siRNA sense strand
acgggactgtgcatgccat

SEQ ID NO: 21 - DNA, 19 bp, Artificial Sequence
  mAmphiregulin siRNA sense strand(control)
cagttgtcactttttatga

SEQ ID NO: 22 - DNA, 21 bp, Artificial Sequence
  mGAPDH-F primer
aggtcggtgtgaacggatttg

SEQ ID NO: 23 - DNA, 23 bp, Artificial Sequence
  mGAPDH-R primer
tgtagaccatgtagttgaggtca

SEQ ID NO: 24 - DNA, 20 bp, Artificial Sequence
  mAREG-F primer
gaggcttcgacaagaaaacg

SEQ ID NO: 25 - DNA, 20 bp, Artificial Sequence
  mAREG-R primer
accaatgtcatttccggtgt

SEQ ID NO: 26 - DNA, 21 bp, Artificial Sequence
  AREG Forward primer
cagtgctgatggatttgaggt

SEQ ID NO: 27 - DNA, 22 bp, Artificial Sequence
  AREG Reverse primer
atagccaggtatttgtggttcg

SEQ ID NO: 28 - DNA, 23 bp, Artificial Sequence
  AREG probe
tgaaccgtcctcgggagccgact

SEQ ID NO: 29 - DNA, 20 bp, Artificial Sequence
  RPL13A Forward primer
gtgtttgacggcatcccacc

SEQ ID NO: 30 - DNA, 20 bp, Artificial Sequence
  RPL13A Reverse primer
taggcttcagacgcacgacc

SEQ ID NO: 31 - DNA, 21 bp, Artificial Sequence
  RPL13A probe
aagcggatggtggttcctgct

SEQ ID NO: 32 - DNA, 19 bp, Artificial Sequence
  TBP Forward primer
caccacagctcttccactc

SEQ ID NO: 33 - DNA, 20 bp, Artificial Sequence
  TBP Reverse primer
atcccagaactctccgaagc

SEQ ID NO: 34 - DNA, 20 bp, Artificial Sequence
  TBP probe
acccttgccgggcaccactc

SEQ ID NO: 35 - RNA, 19 nt, Artificial Sequence
  Amphiregulin siRNA antisense
gcaccugccgcuuuauagg

SEQ ID NO: 36 - RNA, 19 nt, Artificial Sequence
  Amphiregulin siRNA antisense
ccgggagugugcgccgcuc

SEQ ID NO: 37 - RNA, 19 nt, Artificial Sequence
  Amphiregulin siRNA antisense
gcaacucggucucugggac

SEQ ID NO: 38 - RNA, 19 nt, Artificial Sequence
  Amphiregulin siRNA antisense
uucgcagcggcggcgucuc

SEQ ID NO: 39 - RNA, 19 nt, Artificial Sequence
  Amphiregulin siRNA antisense
acagcaccaccggcgccgg

SEQ ID NO: 40 - RNA, 19 nt, Artificial Sequence
  Amphiregulin siRNA antisense
caagagcgacagcaccacc

SEQ ID NO: 41 - RNA, 19 nt, Artificial Sequence
  Amphiregulin siRNA antisense
gagccgaguaucaagagcg

SEQ ID NO: 42 - RNA, 19 nt, Artificial Sequence
  Amphiregulin siRNA antisense
ccugagccgaguaucaaga

SEQ ID NO: 43 - RNA, 19 nt, Artificial Sequence
  Amphiregulin siRNA antisense
guaggugucauugaggucc

SEQ ID NO: 44 - RNA, 19 nt, Artificial Sequence
  Amphiregulin siRNA antisense
acgcuucccagaguaggug

SEQ ID NO: 45 - RNA, 19 nt, Artificial Sequence
  Amphiregulin siRNA antisense
cacgcuucccagaguaggu

SEQ ID NO: 46 - RNA, 19 nt, Artificial Sequence
  Amphiregulin siRNA antisense
aaugguucacgcuucccag

SEQ ID NO: 47 - RNA, 19 nt, Artificial Sequence
  Amphiregulin siRNA antisense
agaaaaugguucacgcuuc

SEQ ID NO: 48 - RNA, 19 nt, Artificial Sequence
  Amphiregulin siRNA antisense
agcacugugguccccagaa

SEQ ID NO: 49 - DNA, 19 bp, Artificial Sequence
  SAMiRNA-Control(human) Sense
cttacgctgagtacttcga

SEQ ID NO: 50 - RNA, 19 nt, Artificial Sequence
  SAMiRNA-Control(human) Antisense
ucgaaguacucagcguaag

SEQ ID NO: 51 - DNA, 25 bp, Artificial Sequence
  Areg Forward primer
agtagtagctgtcactatctttgtc

SEQ ID NO: 52 - DNA, 19 bp, Artificial Sequence
  Areg Reverse primer
cccgttttcttgtcgaagc

SEQ ID NO: 53 - DNA, 23 bp, Artificial Sequence
  Areg probe
cctcgcagctattggcatcggca

SEQ ID NO: 54 - DNA, 22 bp, Artificial Sequence
  Tfrc Forward primer
aaacttgcccaagtattctcag

SEQ ID NO: 55 - DNA, 21 bp, Artificial Sequence
  Tfrc Reverse primer
atgaaaggtatccctccaacc

SEQ ID NO: 56 - DNA, 23 bp, Artificial Sequence
  Tfrc probe
tgccagctggactgcaggcgact

SEQ ID NO: 57 - DNA, 20 bp, Artificial Sequence
  Areg Forward primer
gaggcttcgacaagaaaacg

SEQ ID NO: 58 - DNA, 20 bp, Artificial Sequence
  Areg Reverse primer
accaatgtcatttccggtgt

SEQ ID NO: 59 - DNA, 20 bp, Artificial Sequence
  Gapdh Forward primer
agggtggagccaaaagggtc

SEQ ID NO: 60 - DNA, 20 bp, Artificial Sequence
  Gapdh Reverse primer
ggctaagcagttggtggtgc